European Patent Specification EP 3 169 347 B1, published September 2, 2026. Title: THERAPEUTIC USE OF P75NTR NEUROTROPHIN BINDING PROTEIN. Applicant: Levicept Ltd. The sequence listing filed with the application follows.

SEQUENCE LISTING (32 sequences)

SEQ ID NO: 1 - protein, 460 aa, Artificial Sequence
  Fusion Protein
KEACPTGLYTHSGECCKACNLGEGVAQPCGANQTVCEPCLDSVTFSDVVSATEPCKPCTECVGLQSMSAPCVEADDAVCRCAYGYYQDETTGRCEACRVCEAGSGLVFSCQDKQNTVCEECPDGTYSDEANHVDPCLPCTVCEDTERQLRECTRWADAECEEIPGRWITRSTPPEGSDSTAPSTQEPEAPPEQDLIASTVAGVVTTVMGSSQPVVTRGTTDNDIEGRMDPKSCDKTHTCPPCPAPELLGGPSVFLFPPKPKDTLMISRTPEVTCVVVDVSHEDPEVKFNWYVDGVEVHNAKTKPREEQYNSTYRVVSVLTVLHQDWLNGKEYKCKVSNKALPAPIEKTISKAKGQPREPQVYTLPPSRDELTKNQVSLTCLVKGFYPSDIAVEWESNGQPENNYKTTPPVLDSDGSFFLYSKLTVDKSRWQQGNVFSCSVMHEALHNHYTQKSLSLSPGK

SEQ ID NO: 2 - protein, 462 aa, Artificial Sequence
  Fusion Protein
MEWSWVFLFFLSVTTGVHSKEACPTGLYTHSGECCKACNLGEGVAQPCGANQTVCEPCLDSVTFSDVVSATEPCKPCTECVGLQSMSAPCVEADDAVCRCAYGYYQDETTGRCEACRVCEAGSGLVFSCQDKQNTVCEECPDGTYSDEANHVDPCLPCTVCEDTERQLRECTRWADAECEEIPGRWITRSTPPEGSDSTAPSTQEPEAPPEQDLIASTVAGVVTTVMGGGGEPKSSDKTHTCPPCPAPELLGGPSVFLFPPKPKDTLMISRTPEVTCVVVDVSHEDPEVKFNWYVDGVEVHNAKTKPREEQYNSTYRVVSVLTVLHQDWLNGKEYKCKVSNKALPAPIEKTISKAKGQPREPQVYTLPPSRDELTKNQVSLTCLVKGFYPSDIAVEWESNGQPENNYKTTPPVLDSDGSFFLYSKLTVDKSRWQQGNVFSCSVMHEALHNHYTQKSLSLSPG

SEQ ID NO: 3 - protein, 443 aa, Artificial Sequence
  Fusion protein
KEACPTGLYTHSGECCKACNLGEGVAQPCGANQTVCEPCLDSVTFSDVVSATEPCKPCTECVGLQSMSAPCVEADDAVCRCAYGYYQDETTGRCEACRVCEAGSGLVFSCQDKQNTVCEECPDGTYSDEANHVDPCLPCTVCEDTERQLRECTRWADAECEEIPGRWITRSTPPEGSDSTAPSTQEPEAPPEQDLIASTVAGVVTTVMGGGGEPKSSDKTHTCPPCPAPELLGGPSVFLFPPKPKDTLMISRTPEVTCVVVDVSHEDPEVKFNWYVDGVEVHNAKTKPREEQYNSTYRVVSVLTVLHQDWLNGKEYKCKVSNKALPAPIEKTISKAKGQPREPQVYTLPPSRDELTKNQVSLTCLVKGFYPSDIAVEWESNGQPENNYKTTPPVLDSDGSFFLYSKLTVDKSRWQQGNVFSCSVMHEALHNHYTQKSLSLSPG

SEQ ID NO: 4 - DNA, 1411 bp, Artificial Sequence
  Cloning insert
aagcttgccgccaccatggaatggtcctgggtgttcctgttcttcctgtccgtgaccaccggcgtgcactccaaagaggcttgtcccaccggcctgtacacccactctggcgagtgttgcaaggcctgtaacctgggagaaggcgtggcccagccttgtggcgctaatcagacagtgtgcgagccctgcctggactccgtgaccttctccgatgtggtgtccgccaccgagccttgcaagccctgcacagagtgtgtgggcctgcagtccatgtccgccccttgcgtggaagccgacgacgccgtgtgtagatgcgcctacggctactaccaggacgagacaaccggcagatgcgaggcctgcagagtgtgcgaagctggctctggcctggtgttcagttgtcaagacaagcagaacaccgtgtgcgaggaatgccccgacggcacctactctgacgaggccaatcacgtggacccctgcctgccttgcaccgtgtgtgaagataccgagcggcagctgcgcgagtgcaccagatgggctgatgccgagtgcgaagagatccctggccggtggatcaccagatccacccctccagagggctccgactctaccgctccctctacccaggaacctgaggcccctcctgagcaggacctgatcgcttctacagtggccggcgtcgtgaccacagtgatgggcggaggcggcgagcctaagtcctccgacaagacccacacctgtcccccttgtcctgcccctgaactgctgggcggaccttccgtgtttctgttccccccaaagcccaaggacaccctgatgatctcccggacccccgaagtgacctgcgtggtggtggatgtgtcccacgaggaccctgaagtgaagttcaattggtacgtggacggcgtggaagtgcacaacgccaagaccaagcccagagaggaacagtacaactccacctaccgggtggtgtctgtgctgaccgtgctgcaccaggactggctgaacggcaaagagtacaagtgcaaggtgtccaacaaggccctgccagcccccatcgaaaagaccatctccaaggccaagggccagccccgggaaccccaggtgtacacactgccccctagcagggacgagctgaccaagaaccaggtgtccctgacctgtctcgtgaagggcttctacccctccgatatcgccgtggaatgggagtccaacggccagcctgagaacaactacaagaccaccccccctgtgctggacagcgacggctcattctttctgtactccaagctgacagtggacaagtcccggtggcagcagggcaacgtgttctcctgcagcgtgatgcacgaggctctgcacaaccactacacccagaagtccctgtccctgagccccggctgatgaattc

SEQ ID NO: 5 - protein, 21 aa, Artificial Sequence
  Secretase site
GSSQPVVTRGTTDNDIEGRMD

SEQ ID NO: 6 - protein, 51 aa, Artificial Sequence
  Partial sequence for sequence alignment.
IASTVAGVVTTVMGSSQPVVTRGTTDNLIPVYCSILAAVVVGLVAYIAFKR

SEQ ID NO: 7 - protein, 50 aa, Artificial Sequence
  Partial sequence for sequence alignment
IASTVAGVVTTVMGIPKVDKKVEPKSCDKTHTCPPCPAPELLGGPSVFLF

SEQ ID NO: 8 - protein, 50 aa, Artificial Sequence; identical to SEQ ID NO: 7
  Partial sequence for sequence alignment

SEQ ID NO: 9 - protein, 50 aa, Artificial Sequence
  Partial sequence for sequence alignment
IASTVAGVVTTVMGIPKVDKKVEPKSSDKTHTCPPCPAPELLGGPSVFLF

SEQ ID NO: 10 - protein, 45 aa, Artificial Sequence
  Partial sequence for sequence alignment
IASTVAGVVTTVMGGGGEPKSSDKTHTCPPCPAPELLGGPSVFLF

SEQ ID NO: 11 - protein, 46 aa, Artificial Sequence
  Partial sequence for sequence alignment
IASTVAGVVTTVMGGGGSEPKSSDKTHTCPPCPAPELLGGPSVFLF

SEQ ID NO: 12 - protein, 51 aa, Artificial Sequence
  Partial sequence for sequence alignment
IASTVAGVVTTVMGGGGSGGGGSEPKSSDKTHTCPPCPAPELLGGPSVFLF

SEQ ID NO: 13 - protein, 36 aa, Artificial Sequence
  Partial sequence for sequence alignment
NTKVDKKVEPKSCDKTHTCPPCPAPELLGGPSVFLF

SEQ ID NO: 14 - protein, 427 aa, Homo Sapiens
MGAGATGRAMDGPRLLLLLLLGVSLGGAKEACPTGLYTHSGECCKACNLGEGVAQPCGANQTVCEPCLDSVTFSDVVSATEPCKPCTECVGLQSMSAPCVEADDAVCRCAYGYYQDETTGRCEACRVCEAGSGLVFSCQDKQNTVCEECPDGTYSDEANHVDPCLPCTVCEDTERQLRECTRWADAECEEIPGRWITRSTPPEGSDSTAPSTQEPEAPPEQDLIASTVAGVVTTVMGSSQPVVTRGTTDNLIPVYCSILAAVVVGLVAYIAFKRWNSCKQNKQGANSRPVNQTPPPEGEKLHSDSGISVDSQSLHDQQPHTQTASGQALKGDGGLYSSLPPAKREEVEKLLNGSAGDTWRHLAGELGYQPEHIDSFTHEACPVRALLASWATQDSATLDALLAALRRIQRADLVESLCSESTATSPV

SEQ ID NO: 15 - protein, 250 aa, Homo Sapiens
MGAGATGRAMDGPRLLLLLLLGVSLGGAKEACPTGLYTHSGECCKACNLGEGVAQPCGANQTVCEPCLDSVTFSDVVSATEPCKPCTECVGLQSMSAPCVEADDAVCRCAYGYYQDETTGRCEACRVCEAGSGLVFSCQDKQNTVCEECPDGTYSDEANHVDPCLPCTVCEDTERQLRECTRWADAECEEIPGRWITRSTPPEGSDSTAPSTQEPEAPPEQDLIASTVAGVVTTVMGSSQPVVTRGTTDN

SEQ ID NO: 16 - protein, 221 aa, Homo Sapiens
KEACPTGLYTHSGECCKACNLGEGVAQPCGANQTVCEPCLDSVTFSDVVSATEPCKPCTECVGLQSMSAPCVEADDAVCRCAYGYYQDETTGRCEACRVCEAGSGLVFSCQDKQNTVCEECPGTYSDEANHVDPCLPCTVCEDTERQLRECTRWADAECEEIPGRWITRSTPPEGSDSTAPSTQEPEAPPEQDLIASTVAGVVTTVMGSSQPVVTRGTTDN

SEQ ID NO: 17 - protein, 13 aa, Homo Sapiens
CAYGYYQDETTGR

SEQ ID NO: 18 - protein, 49 aa, Homo Sapiens
VCEAGSGLVFSCQDKQNTVCEECPGGTYSDEANHVDPCLPCTVCEDTER

SEQ ID NO: 19 - protein, 15 aa, Homo Sapiens
VCEAGSGLVFSCQDK

SEQ ID NO: 20 - protein, 12 aa, Homo Sapiens
WADAECEEIPGR

SEQ ID NO: 21 - protein, 17 aa, Homo Sapiens
LDSVTSDVVSATEPCKP

SEQ ID NO: 22 - protein, 698 aa, Homo Sapiens
MRLAVGALLVCAVLGLCLAVPDKTVRWCAVSEHEATKCQSFRDHMKSVIPSDGPSVACVKKASYLDCIRAIAANEADAVTLDAGLVYDAYLAPNNLKPVVAEFYGSKEDPQTFYYAVAVVKKDSGFQMNQLRGKKSCHTGLGRSAGWNIPIGLLYCDLPEPRKPLEKAVANFFSGSCAPCADGTDFPQLCQLCPGCGCSTLNQYFGYSGAFKCLKDGAGDVAFVKHSTIFENLANKADRDQYELLCLDNTRKPVDEYKDCHLAQVPSHTVVARSMGGKEDLIWELLNQAQEHFGKDKSKEFQLFSSPHGKDLLFKDSAHGFLKVPPRMDAKMYLGYEYVTAIRNLREGTCPEAPTDECKPVKWCALSHHERLKCDEWSVNSVGKIECVSAETTEDCIAKIMNGEADAMSLDGGFVYIAGKCGLVPVLAENYNKSDNCEDTPEAGYFAVAVVKKSASDLTWDNLKGKKSCHTAVGRTAGWNIPMGLLYNKINHCRFDEFFSEGCAPGSKKDSSLCKLCMGSGLNLCEPNNKEGYYGYTGAFRCLVEKGDVAFVKHQTVPQNTGGKNPDPWAKNLNEKDYELLCLDGTRKPVEEYANCHLARAPNHAVVTRKDKEACVHKILRQQQHLFGSNVTDCSGNFCLFRSETKDLLFRDDTVCLAKLHDRNTYEKYLGEEYVKAVGNLRKCSTSSLLEACTFRRP

SEQ ID NO: 23 - protein, 609 aa, Homo Sapiens [sequence omitted]

SEQ ID NO: 24 - protein, 212 aa, Homo Sapiens
GGPSVFLFPPKPKDTLMISRTPEVTCVVVDVSHEDPEVKFNWYVDGVEVHNAKTKPREEQYDSTYRVVSVLTVLHQDWLNGKEYKCKVSNKALPAPIEKTISKAKGQPREPQVYTLPPSREEMTKNQVSLTCLVKGFYPSDIAVEWESNGQPENNYKTTPPVLDSDGSFFLYSKLTVDKSRWQQGNVFSCSVMHEALHNHYTQKSLSLSPGK

SEQ ID NO: 25 - protein, 326 aa, Homo Sapiens
ASTKGPSVFPLAPCSRSTSESTAALGCLVKDYFPEPVTVSWNSGALTSGVHTFPAVLQSSGLYSLSSVVTVTSSNFGTQTYTCNVDHKPSNTKVDKTVERKCCVECPPCPAPPVAGPSVFLFPPKPKDTLMISRTPEVTCVVVDVSHEDPEVQFNWYVDGMEVHNAKTKPREEQFNSTFRVVSVLTVVHQDWLNGKEYKCKVSNKGLPAPIEKTISKTKGQPREPQVYTLPPSREEMTKNQVSLTCLVKGFYPSDIAVEWESNGQPENNYKTTPPMLDSDGSFFLYSKLTVDKSRWQQGNVFSCSVMHEALHNHYTQKSLSLSPGK

SEQ ID NO: 26 - protein, 165 aa, Homo Sapiens
CYTLLLLTTPSWVLSQVTLKESGPVLVKPTETLTLTCTVSGFSLSNAKMGVSWIRQPPGKALEWLAHIFSNDEKSYSTSLKSRLTISKDTSKSQVVLTMTNMDPVDTATYYCARIFTITYSNYVLQYYYYMDVWGKGTTVTVSSASTKGPSVFPLAPCSRSTSGG

SEQ ID NO: 27 - protein, 217 aa, Homo Sapiens
APEFLGGPSVFLFPPKPKDTLMISRTPEVTCVVVDVSQEDPEVQFNWYVDGVEVHNAKTKPREEQFNSTYRVVSVLTVLHQDWLNGKEYKCKVSNKGLPSSIEKTISKAKGQPREPQVYTLPPSQEEMTKNQVSLTCLVKGFYPSDIAVEWESNGQPENNYKTTPPVLDSDGSFFLYSKLTVDKSRWQEGNVFSCSVMHEALHNHYTQKSLSLSLGK

SEQ ID NO: 28 - protein, 209 aa, Artificial
  Engineered Fc Fragment
GGPSVFLFPPKPKDTLYITREPEVTCVVVDVSHEDPEVKFNWYVDGVEVHNAKTKPREEQYNSTYRVVSVLTVLHQDWLNGKEYKCKVSNKALPAPIEKTISKAKGQPREPQVYTLPPSRDELTKNQVSLTCLVKGFYPSDIAVEWESNGQPENNYKTTPPVLDSDGSFFLYSKLTVDKSRWQQGNVFSCSVMHEALHNHYTQKSLSLS

SEQ ID NO: 29 - protein, 225 aa, Artificial
  Engineered Fc Fragment
THTCPPCPAPEFEGGPSVFLFPPKPKDTLMISRTPEVTCVVVDVSHEDPEVKFNWYVDGVEVHNAKTKPREEQYNSTYRVVSVLTVLHQDWLNGKEYKCKVSNKALPASIEKTISKAKGQPREPQVYTLPPSREEMTKNQVSLTCLVKGFYPSDIAVEWESNGQPENNYKTTPPVLDSDGSFFLYSKLTVDKSRWQQGNVFSCSVMHEALHNHYTQKSLSLSPGK

SEQ ID NO: 30 - protein, 5 aa, Artificial
  Linker peptide
GGGGS

SEQ ID NO: 31 - protein, 5 aa, Artificial
  Linker peptide
EAAAK

SEQ ID NO: 32 - protein, 5 aa, Artificial
  Linker peptide
GGGGS